European Patent Specification EP 4 127 152 B1, published August 12, 2026. Title: METHODS, COMPOSITIONS, AND KITS FOR IDENTIFYING REGIONS OF GENOMIC DNA BOUND TO A PROTEIN. Applicant: Altius Institute for Biomedical Sciences The Brigham and Women's Hospital, Inc. Stamatoyannopoulos, John A. Stergachis, Andrew B. The sequence listing filed with the application follows.

SEQUENCE LISTING (5 sequences)

SEQ ID NO: 1 - protein, 281 aa, H. influenzae
MANQNTFKQAPLPFIGQKRMFLKQFEQILNENISDNGEGWTILDTFGGSGLLSHTAKRLKPKARVIYNDFDGYAERLAHIDDINQLRAELYSVVGNATSKNKRMTKDCKAECIRIIQNFKGYKDLNCLASWLLFSGQQVATLDDLFQHNFWHCIRQSDYPKADGYLDGVEIVKESFHTLLPKFSNDPKALFVLDPPYLCTKQESYKQATYFDLIDFLRLVNITRPPYVFFSSTKSEFIRFVNYMLEDKVDNWQAFENAKRITVNAKLNYQVAYEDNLVYKF

SEQ ID NO: 2 - protein, 296 aa, H. influenzae
MSEYLEYQNAIEGKTMANKKTFKQAPLPFIGQKRMFLKHVEIVLNKHIDGEGEGWTIVDVFGGSGLLSHTAKQLKPKATVIYNDFDGYAERLNHIDDINRLRQIIFNCLHGIIPKNGRLSKEIKEEIINKINDFKGYKDLNCLASWLLFSGQQVGSVEALFAKDFWNCVRQSDYPTAEGYLDGIEVISESFHKLIPRYQNQDKVLLLLDPPYLCTRQESYKQATYFDLIDFLRLINLTKPPYIFFSSTKSEFIRYLNYMQESKTDNWRAFENYKRIVVKASASKDGIYEDNMIYKF

SEQ ID NO: 3 - protein, 317 aa, Bibersteinia trehalosi
MKKTLTALAVASLASATQTKQQASKQASKQASKQASKECEMAKVFKQAPLPFIGQKRMFLKHFEQVLAHIPDDGNGWTIVDVFGGSGLLSHTAKRLKPKARVIYNDYDNYSERLQHIDDINRLRRIIADLMADTPKYKRLDNAKKLQIIEAIEAFQGYKDLHILCSWLAFSGQQVSSFDELYKQNFWHCIRQSDYLTADGYLDGVEIVRESFHQLVPRFTGQPNTLLVLDPPYLCTHQESYKQERYFDLVDFLRLIHLTKPPYVFFSSTKSEFVRFIDAMVEDKWDNWQAFDDAQRIVVQTSASYNGKYEDNMVYKF

SEQ ID NO: 4 - protein, 227 aa, Escherichia coli
MSRFILGDCVRVMATFPDNAVDFILTDPPYLVGFRDRSGRTIAGDVNDDWLQPASNEMYRVLKKDALMVSFYGWNRIDRFMAAWKRAGFSVVGHLVFTKNYTSKAAYVGYRHECAYILAKGRPALPQKPLPDVLGWKYSGNRHHPTEKPVTSLQPLIESFTHPNAIVLDPFAGSGSTCVAALQSGRRYIGIELLEQYHRAGQQRLAAVQRAMQQGAANDNWFEPEAA

SEQ ID NO: 5 - DNA, 16 bp, Artificial sequence
  synthetic sequence
agatcggaagagcgtc